European Patent Application EP 4 417 684 A1, published August 21, 2024. Title: Bacteria modified to express heterogeneous Tat proteins. Applicant: Ajinomoto Co., Inc. The sequence listing filed with the application follows.

SEQUENCE LISTING (93 sequences)

SEQ ID NO: 1 - DNA, 125 bp, Lactococcus lactis
  source 1..125: mol_type = genomic DNA
ctctgtaaaagctgtcagtagacagtttttttaataagttaaagaaaagatgtaatttttctttgtactcgaaattttctattcaatttgatataattatattaatactgaatatttaggagaag

SEQ ID NO: 2 - DNA, 36 bp, synthetic construct
  misc_feature 1..36: note = primer
  source 1..36: mol_type = other DNA
ttacagctccagatctctctgtaaaagctgtcagta

SEQ ID NO: 3 - DNA, 40 bp, synthetic construct
  misc_feature 1..40: note = primer
  source 1..40: mol_type = other DNA
gaactagtggtaccgcatgccttctcctaaatattcagta

SEQ ID NO: 4 - DNA, 354 bp, Corynebacterium glutamicum
  source 1..354: mol_type = genomic DNA
atgcccactctcggaccatgggaaatcgcgatcattgtcctgctgatcattctgctgttcggcgcgaagaagctgcctgatgcagctcgttccatcggccgttccatgcgcatcttcaagtctgaagtcaaagaaatgaacaaggacggcgataccccagaacaacaacagcagcagcctcagcagcagcagcagattgcgcccaaccagatcgaggctcctcagccagttcagcagccagcgcaacagtcaaactttgagcagcactaccagggccagcaggttcagcagcctcagaaccctcagacccctgactaccgtcagaactacgaggatccaaaccgcacctcctaa

SEQ ID NO: 5 - DNA, 471 bp, Corynebacterium glutamicum
  source 1..471: mol_type = genomic DNA
atgttttctagcgtgggttggggagagatcttcctcttagtcgttgtgggccttgttgtcatcggcccggaacggttgcctcgtttgatccaggacgcacgcgctgcgctgctcgctgcacgtaccgctatcgacaatgcaaagcagtcgttggacagtgattttggttcggaatttgatgaaatccgaaagccactaacccaggttgcacagtacagccggatgagccccaagacggccatcactaaggcgttgtttgataatgattcctcgttcctggatgactttgatccaaagaagatcatggccgaaggaacagaaggcgaagctcagcgccacaagcaggcagctgacaacaatgcgaatgtggtggaacgtccagctgatggttccaccgcacgcccaacgcaaaacgatccaaaagacggcccgaattactcaggcggcgtctcttggaccgatattatttag

SEQ ID NO: 6 - DNA, 945 bp, Corynebacterium glutamicum
  source 1..945: mol_type = genomic DNA
atgtccattgttgagcacatcaaagagtttcgacgccgacttctcatcgctctggcgggcatcctcgtgggcaccattatcggctttatttggtacgatttctcattttggcagatccccactttgggcgagctgctgagggatccgtactgttctttgcctgctgaatcccgctgggccatgagcgactcagaggaatgtcgactgctcgcaaccggcccgtttgatccattcatgcttcgccttaaagtagcggcgttggtgggtatggttcttggctcacccgtgtggctgagccagctgtggggctttatcaccccaggtttgatgaagaatgagcgccgttacaccgcaatcttcgtcacgattgctgttgtgctgtttgtcggcggtgctgttcttgcgtacttcgtcgttgcatatggtttggagttcctccttaccattggtggagacacccaggcagcggccctgactggtgataagtacttcggattcttgctcgcgttgttggcgattttcggcgtgagcttcgaagttccactggtgatcggcatgctcaacattgtgggtatcttgccctacgatgccattaaagataagcgacgcatgatcatcatgattttgttcgtgttcgctgctttcatgacacccggccaggatcctttcaccatgttggtgttggcgctttcactcaccgttctggtggagcttgccctgcagttctgtcgcttcaacgacaaacgccgggacaagaagcgcccagaatggcttgatggcgatgacctctctgcatcaccactggatacttctgctggtggagaagatgctccaagcccagtcgaaaccccagaggcggtggagccttcgcggatgctgaacccaagtggggaggcgtcgataagctataaacccgggcgcgccgacttcggtgacgtgctctag

SEQ ID NO: 7 - DNA, 1790 bp, synthetic construct
  source 1..1790: mol_type = other DNA
atgccaacacttggtccatgggaaattgctattattgtattattgattattttactttttggcgcaaaaaaattgccagatgctgcgcgttcaattggacgaagtatgcgtatctttaaaagtgaggtaaaggaaatgaataaagatggtgacacacctgaacaacaacaacaacaaccacaacaacaacaacaaattgcaccaaatcaaattgaggctcctcaaccagtacaacagcctgctcaacaaagtaattttgaacaacattatcaaggccaacaagtccaacaaccacaaaacccacaaacgccagattatcgtcaaaattatgaagacccaaatcgaacgtcataaaggagaaggcatgagtattgtggaacatattaaagagtttcgacgccgtttacttattgcacttgcggggattcttgttggaacgattatcggattcatctggtatgattttagtttctggcaaattcctacattgggagagttacttcgtgacccatattgtagtcttcctgccgagtcacgctgggctatgtctgattcagaagaatgccgtttattagcaaccgggccatttgatcctttcatgttacgtttgaaagtggctgcacttgtaggcatggttttgggctctccagtctggttatctcaattatggggttttatcactccaggtttgatgaaaaatgaacgtcgttacactgcaatatttgttacaattgcagttgtcttatttgtgggaggagcggtattagcatattttgtcgtagcatatggtttagaatttcttcttactatcggtggagatacacaagcggcggcattaacgggagataaatattttggtttcttgcttgctttgcttgctatttttggcgtgagttttgaagtacctcttgttattgggatgttgaatattgtcggaatcttaccatatgacgcaattaaagataaacgtcgaatgattatcatgatattgttcgtatttgccgcatttatgactccaggacaggatccttttactatgttggttttagctttatcattaacggttcttgttgaattggcattacaattctgtcgatttaatgataaacgtcgtgataagaaaagacctgagtggcttgatggtgatgatcttagtgcatcaccacttgacacctcagctggaggagaggatgcaccatctcctgttgaaacgccagaagcagtagaaccttcacgaatgttaaatccatctggagaagcatctatatcatacaaacctggtcgtgctgatttcggtgatgttctttgaaggagaaggcatgttttcatctgtgggatggggtgaaattttccttcttgttgtagtaggtcttgtagtaattggaccagaacgccttccacgccttatccaggatgcgcgtgcagctttgttagccgcacgtacagctattgacaatgccaaacaatcattagattctgatttcggatcagagttcgatgaaattagaaaaccacttacacaagttgctcaatattctagaatgtctccaaaaacagcaataactaaagccttatttgacaatgattcttcatttttagacgattttgacccaaagaaaattatggcagaaggcaccgaaggagaagcacaacgtcataaacaagcagcagacaataatgcaaatgtcgtagaacgccctgcagacggtagtacagctcgtcctacacaaaacgatccaaaagatggcccaaattatagtgggggtgtttcatggactgatatcatttaa

SEQ ID NO: 8 - DNA, 31 bp, synthetic construct
  misc_feature 1..31: note = primer
  source 1..31: mol_type = other DNA
actagtatgccaacacttggtccatgggaaa

SEQ ID NO: 9 - DNA, 31 bp, synthetic construct
  misc_feature 1..31: note = primer
  source 1..31: mol_type = other DNA
aagcttttaaatgatatcagtccatgaaaca

SEQ ID NO: 10 - DNA, 117 bp, Escherichia coli
  source 1..117: mol_type = genomic DNA
atgaacaataacgatctctttcaggcatcacgtcggcgttttctggcacaactcggcggcttaaccgtcgccgggatgctggggccgtcattgttaacgccgcgacgtgcgactgcg

SEQ ID NO: 11 - DNA, 468 bp, Homo sapiens
  source 1..468: mol_type = other DNA
atggctgccggatctattaccacgctcccggcgctcccggaagacggtggaagcggcgccttcccacctggccacttcaaagacccgaaacgtctgtattgtaaaaatggcggttttttcctccgcatccacccagatggtcgcgtcgatggtgtccgcgaaaagtccgacccacacatcaagctgcaactgcaagcagaggaacgtggcgtcgtgagcatcaagggcgtgtgcgcaaaccgctatctggccatgaaggaggatggtcgccttcttgcatccaaatgcgtgaccgatgaatgcttcttctttgaacggctggagtccaacaattacaacacctaccgctcccgcaagtatacctcctggtatgtcgccctgaaacgcacgggacaatataaactgggttccaagaccggtcctggccaaaaggcgattcttttcctcccaatgtccgcgaagtcttga

SEQ ID NO: 12 - DNA, 582 bp, synthetic construct
  source 1..582: mol_type = other DNA
atgaataataatgatttatttcaagcatctagacgacgatttttggctcaattaggcggtttgacagttgctgggatgttgggtccttcattattgactcctcgtcgtgccaccgcagcagcaggaagtatcaccactcttcctgcattacctgaggatggtggatctggagcttttccaccaggacattttaaagatccaaaacgtttgtattgtaaaaacggaggattttttttacgtatccatccagacggacgtgtcgatggagttcgagagaagtcagatccacatattaaattacaattacaggcagaggaaagaggagttgtttctattaaaggagtttgtgcaaatcgttatttagctatgaaagaagatggtcgtttacttgcttctaaatgtgtcactgacgaatgtttcttctttgaaagattggaatctaataattacaatacctatcgttcacgtaaatatacttcatggtatgttgctttaaaacgcactggtcaatataaacttgggtctaagacaggtcctgggcaaaaagctattttatttcttccaatgtcagcgaaaagttaa

SEQ ID NO: 13 - DNA, 31 bp, synthetic construct
  misc_feature 1..31: note = primer
  source 1..31: mol_type = other DNA
actagtatgaataataatgatttatttcaag

SEQ ID NO: 14 - DNA, 31 bp, synthetic construct
  misc_feature 1..31: note = primer
  source 1..31: mol_type = other DNA
aagcttttaacttttcgctgacattggaaga

SEQ ID NO: 15 - DNA, 354 bp, Corynebacterium glutamicum
  source 1..354: mol_type = other DNA
atgccaacacttggtccatgggaaattgctattattgtattattgattattttactttttggcgcaaaaaaattgccagatgctgcgcgttcaattggacgaagtatgcgtatctttaaaagtgaggtaaaggaaatgaataaagatggtgacacacctgaacaacaacaacaacaaccacaacaacaacaacaaattgcaccaaatcaaattgaggctcctcaaccagtacaacagcctgctcaacaaagtaattttgaacaacattatcaaggccaacaagtccaacaaccacaaaacccacaaacgccagattatcgtcaaaattatgaagacccaaatcgaacgtcataa

SEQ ID NO: 16 - DNA, 471 bp, Corynebacterium glutamicum
  source 1..471: mol_type = other DNA
atgttttcatctgtgggatggggtgaaattttccttcttgttgtagtaggtcttgtagtaattggaccagaacgccttccacgccttatccaggatgcgcgtgcagctttgttagccgcacgtacagctattgacaatgccaaacaatcattagattctgatttcggatcagagttcgatgaaattagaaaaccacttacacaagttgctcaatattctagaatgtctccaaaaacagcaataactaaagccttatttgacaatgattcttcatttttagacgattttgacccaaagaaaattatggcagaaggcaccgaaggagaagcacaacgtcataaacaagcagcagacaataatgcaaatgtcgtagaacgccctgcagacggtagtacagctcgtcctacacaaaacgatccaaaagatggcccaaattatagtgggggtgtttcatggactgatatcatttaa

SEQ ID NO: 17 - DNA, 945 bp, Corynebacterium glutamicum
  source 1..945: mol_type = other DNA
atgagtattgtggaacatattaaagagtttcgacgccgtttacttattgcacttgcggggattcttgttggaacgattatcggattcatctggtatgattttagtttctggcaaattcctacattgggagagttacttcgtgacccatattgtagtcttcctgccgagtcacgctgggctatgtctgattcagaagaatgccgtttattagcaaccgggccatttgatcctttcatgttacgtttgaaagtggctgcacttgtaggcatggttttgggctctccagtctggttatctcaattatggggttttatcactccaggtttgatgaaaaatgaacgtcgttacactgcaatatttgttacaattgcagttgtcttatttgtgggaggagcggtattagcatattttgtcgtagcatatggtttagaatttcttcttactatcggtggagatacacaagcggcggcattaacgggagataaatattttggtttcttgcttgctttgcttgctatttttggcgtgagttttgaagtacctcttgttattgggatgttgaatattgtcggaatcttaccatatgacgcaattaaagataaacgtcgaatgattatcatgatattgttcgtatttgccgcatttatgactccaggacaggatccttttactatgttggttttagctttatcattaacggttcttgttgaattggcattacaattctgtcgatttaatgataaacgtcgtgataagaaaagacctgagtggcttgatggtgatgatcttagtgcatcaccacttgacacctcagctggaggagaggatgcaccatctcctgttgaaacgccagaagcagtagaaccttcacgaatgttaaatccatctggagaagcatctatatcatacaaacctggtcgtgctgatttcggtgatgttctttga

SEQ ID NO: 18 - DNA, 354 bp, Corynebacterium glutamicum
  source 1..354: mol_type = other DNA
atgccgaccctgggcccgtgggaaatcgccatcatcgtgctgctgatcatcctgctgttcggcgccaagaagctgccggacgccgcccgctccatcggccgctccatgcgcatcttcaagtccgaagtgaaggagatgaacaaggacggcgacaccccggaacagcagcagcagcagccgcagcagcagcagcagatcgccccgaaccagatcgaagccccgcagccggtgcagcagccggcccagcagtccaacttcgagcagcactaccagggccagcaggtgcagcagccgcagaacccgcagaccccggactaccgccagaactacgaggacccgaaccgcacctcctga

SEQ ID NO: 19 - DNA, 471 bp, Corynebacterium glutamicum
  source 1..471: mol_type = other DNA
atgttctcctccgtgggctggggcgaaatcttcctgctagtggtggtgggcctggtggtgatcggcccggaacgcctgccgcgcctgatccaggacgcccgcgccgccctgctggccgcccgcaccgccatcgacaacgccaagcagtccctggactccgacttcggctccgagttcgacgaaatccgcaagccgctgacccaggtggcccagtactcccgcatgtccccgaagaccgccatcaccaaggccctgttcgacaacgactcctccttcctggacgacttcgacccgaagaagatcatggccgaaggcaccgagggcgaagcccagcgccacaagcaggccgccgacaacaacgccaacgtggtggaacgcccggccgacggctccaccgcccgcccgacccagaacgacccgaaggacggcccgaactactccggcggcgtgtcctggaccgacatcatctga

SEQ ID NO: 20 - DNA, 945 bp, Corynebacterium glutamicum
  source 1..945: mol_type = other DNA
atgtccatcgtggaacacatcaaggagttccgccgccgcctgctgatcgccctggccggcatcctggtgggcaccatcatcggcttcatctggtacgacttctccttctggcagatcccgaccctgggcgaactgctgcgcgacccgtactgctccctgccggccgaatcccgctgggccatgtccgactccgaggaatgccgcctgctggccaccggcccgttcgacccgttcatgctgcgcctgaaggtggccgccctggtgggcatggtgctgggctccccggtgtggctgtcccagctgtggggcttcatcaccccgggcctgatgaagaacgaacgccgctacaccgccatcttcgtgaccatcgccgtggtgctgttcgtgggcggcgccgtgctggcctacttcgtggtggcctacggcctggagttcctgctgaccatcggcggcgacacccaggccgccgccctgaccggcgacaagtacttcggcttcctgctggccctgctggccatcttcggcgtgtccttcgaagtgccgctggtgatcggcatgctgaacatcgtgggcatcctgccgtacgacgccatcaaggacaagcgccgcatgatcatcatgatcctgttcgtgttcgccgccttcatgaccccgggccaggacccgttcaccatgctggtgctggccctgtccctgaccgtgctagtggaactggccctgcagttctgccgcttcaacgacaagcgccgcgacaagaagcgcccggaatggctggacggcgacgacctgtccgcctccccgctggacacctccgccggcggcgaagacgccccgtccccggtggaaaccccggaggccgtggaaccgtcccgcatgctgaacccgtccggcgaagcctccatctcctacaagccgggccgcgccgacttcggcgacgtgctgtga

SEQ ID NO: 21 - DNA, 354 bp, Corynebacterium glutamicum
  source 1..354: mol_type = other DNA
atgcctactttgggtccatgggagatcgcaataatagtcttactaattatattgttatttggagcaaaaaaacttccagatgcagcgagatctataggtcgtagtatgcgaatatttaaaagtgaagtcaaagagatgaataaggacggtgatacacctgaacaacaacaacaacagccacaacaacaacaacaaatcgctccaaatcaaatagaagcaccacaaccagttcaacaacctgcgcaacaatctaatttcgaacaacattatcagggccaacaagtgcagcaaccacaaaatcctcaaacacctgattatagacaaaattatgaagatccaaatagaacaagttga

SEQ ID NO: 22 - DNA, 471 bp, Corynebacterium glutamicum
  source 1..471: mol_type = other DNA
atgttttcatctgttggatggggagaaatttttttattagttgttgtgggtttggtagtgattggcccagaaagacttccaagattaatacaagatgcacgagctgctttgctagcagctcgtacagcaatagacaatgcaaaacaaagtcttgatagtgatttcggatcagaatttgatgaaattcgtaaacctcttacacaagttgcacaatactcacgaatgagtccaaaaactgctattactaaagcattgtttgataatgattcttcatttcttgatgactttgacccaaaaaagataatggctgaaggtactgaaggtgaagcacaaagacacaaacaagctgctgataataatgcgaatgtggtggaaagacctgcagatggttctacggcacgtccaacacaaaatgatccaaaagatggtccaaattacagtggtggagttagttggacagacattatatag

SEQ ID NO: 23 - DNA, 945 bp, Corynebacterium glutamicum
  source 1..945: mol_type = other DNA
atgagtatcgtagaacatattaaggaatttcgtagaagattgctaattgcacttgcaggaatcttagttggtactattattggatttatttggtacgatttttcattctggcaaattcctactctaggtgagttattacgtgatccatattgtagtttaccagctgagtctcgttgggcaatgtctgattctgaagaatgtcgtttactagcaacaggtccttttgatccatttatgttacgacttaaagtagcagcacttgtgggaatggtcttaggaagtcctgtttggttatctcagttgtggggttttataacgccaggcctaatgaaaaatgaacgtcgttatactgcgattttcgttacaattgcagttgttttgtttgtaggtggcgcagtcttagcatattttgtggtagcttatggtcttgagttcttacttactattggtggtgacacgcaagctgcagcattaacaggtgataaatattttggttttttacttgcattattagcaatttttggcgtgtctttcgaagtgcctttagtaattggtatgttaaatattgtgggcattttaccttatgatgcaataaaagacaaaagacgtatgatcattatgattttatttgtttttgctgctttcatgacgccaggtcaggatccatttactatgttagtattagctttaagtttaacagtattagtagaattagcattacaattctgtcgttttaatgataaacgtagagacaaaaagcgtcctgaatggttagatggagatgatctttctgcatcacctttagatacaagtgcaggcggagaagatgcgccatcacctgttgaaacacctgaagctgtagaaccttcacgtatgcttaatcctagtggagaagcatcaatttcatataaaccaggtcgagcagattttggtgacgtattgtag

SEQ ID NO: 24 - protein, 117 aa, Corynebacterium glutamicum
MPTLGPWEIAIIVLLIILLFGAKKLPDAARSIGRSMRIFKSEVKEMNKDGDTPEQQQQQPQQQQQIAPNQIEAPQPVQQPAQQSNFEQHYQGQQVQQPQNPQTPDYRQNYEDPNRTS

SEQ ID NO: 25 - protein, 156 aa, Corynebacterium glutamicum
MFSSVGWGEIFLLVVVGLVVIGPERLPRLIQDARAALLAARTAIDNAKQSLDSDFGSEFDEIRKPLTQVAQYSRMSPKTAITKALFDNDSSFLDDFDPKKIMAEGTEGEAQRHKQAADNNANVVERPADGSTARPTQNDPKDGPNYSGGVSWTDII

SEQ ID NO: 26 - protein, 314 aa, Corynebacterium glutamicum
MSIVEHIKEFRRRLLIALAGILVGTIIGFIWYDFSFWQIPTLGELLRDPYCSLPAESRWAMSDSEECRLLATGPFDPFMLRLKVAALVGMVLGSPVWLSQLWGFITPGLMKNERRYTAIFVTIAVVLFVGGAVLAYFVVAYGLEFLLTIGGDTQAAALTGDKYFGFLLALLAIFGVSFEVPLVIGMLNIVGILPYDAIKDKRRMIIMILFVFAAFMTPGQDPFTMLVLALSLTVLVELALQFCRFNDKRRDKKRPEWLDGDDLSASPLDTSAGGEDAPSPVETPEAVEPSRMLNPSGEASISYKPGRADFGDVL

SEQ ID NO: 27 - DNA, 117 bp, Escherichia coli
  source 1..117: mol_type = other DNA
atgaataataatgatttatttcaagcatctagacgacgatttttggctcaattaggcggtttgacagttgctgggatgttgggtccttcattattgactcctcgtcgtgccaccgca

SEQ ID NO: 28 - DNA, 117 bp, Escherichia coli
  source 1..117: mol_type = other DNA
atgaacaacaacgacctgttccaggcctcccgccgccgcttcctggcccagctgggcggcctgaccgtggccggcatgctgggcccgtccctgctgaccccgcgccgcgccaccgcc

SEQ ID NO: 29 - DNA, 117 bp, Escherichia coli
  source 1..117: mol_type = other DNA
atgaacaataatgacttatttcaagcttcacgtcgtcgtttcttggcacaattgggtggtttgacagttgcaggtatgcttggtccaagtttgttgactccaagacgtgcaactgca

SEQ ID NO: 30 - protein, 324 aa, Escherichia coli
MANMFALILVIATLVTGILWCVDKFFFAPKRRERQAAAQAAAGDSLDKATLKKVAPKPGWLETGASVFPVLAIVLIVRSFIYEPFQIPSGSMMPTLLIGDFILVEKFAYGIKDPIYQKTLIETGHPKRGDIVVFKYPEDPKLDYIKRAVGLPGDKVTYDPVSKELTIQPGCSSGQACENALPVTYSNVEPSDFVQTFSRRNGGEATSGFFEVPKNETKENGIRLSERKETLGDVTHRILTVPIAQDQVGMYYQQPGQQLATWIVPPGQYFMMGDNRDNSADSRYWGFVPEANLVGRATAIWMSFDKQEGEWPTGLRLSRIGGIH

SEQ ID NO: 31 - protein, 184 aa, Bacillus subtilis
MKSENVSKKKSILEWAKAIVIAVVLALLIRNFIFAPYVVDGDSMYPTLHNRERVFVNMTVKYIGEFDRGDIVVLNGDDVHYVKRIIGLPGDTVEMKNDQLYINGKKVDEPYLAANKKRAKQDGFDHLTDDFGPVKVPDNKYFVMGDNRRNSMDSRNGLGLFTKKQIAGTSKFVFYPFNEMRKTN

SEQ ID NO: 32 - protein, 193 aa, Bacillus subtilis
MTEEKNTNTEKTAKKKTNTYLEWGKAIVIAVLLALLIRHFLFEPYLVEGSSMYPTLHDGERLFVNKTVNYIGELKRGDIVIINGETSKIHYVKRLIGKPGETVQMKDDTLYINGKKVAEPYLSKNKKEAEKLGVSLTGDFGPVKVPKGKYFVMGDNRLNSMDSRNGLGLIAEDRIVGTSKFVFFPFNEMRQTK

SEQ ID NO: 33 - protein, 262 aa, Corynebacterium glutamicum
MTDFSSASNADDSTQDGRPGRRAGKSKKESKPTPWYIEIPVVVVLTLALIFVLQTFVGRMYMIPSGSMEPTLHGCEGCTGDRILVEKVSYYFTDPEPGDVVVFKGTDSWNVGFTTQRSDNSVIRGLQNLGSYVGLVAPDENDLVKRIIATGGQTVSCQAGDPGIMVDGKEVDDSYTLQPAQFPIDETSGSTECGGNYFGPITVPDGNYFMMGDNRTNSMDSRYHLGDQYQGTIPEENIKGKVQAIILPFSRIGGVDDPAIKG

SEQ ID NO: 34 - protein, 208 aa, Lactococcus lactis
MMKFLKEWGLFIFIIAAVLLSRVFIWSLVVVDGHSMDPTLADKERLVIVRTTKINRFDIVVAKENAADGSTKDIVKRVVGMPGDTIKFDHDQLTINNKVYPENYLKDYQKQLADGQLEKTYGNYPLTKALTDQNRSLFVSLAQSTKAFTTDSTGNPTFTVKVPDGQYFLMGDNRVVSQDSRAVGSFKRSAIIGEAKLRVWPLNKISFF

SEQ ID NO: 35 - DNA, 213 bp, Bacillus subtilis
  source 1..213: mol_type = genomic DNA
atgttttcaaacattggaataccgggcttgattctcatcttcgtcatcgccctcattatttttggcccttccaagctgccggaaatcgggcgtgccgccggacggacactgctggaatttaaaagcgccacaaaatcacttgtgtctggtgatgaaaaagaagagaaatcagctgagctgacagcggtaaagcaggacaaaaacgcgggctga

SEQ ID NO: 36 - DNA, 729 bp, Bacillus subtilis
  source 1..729: mol_type = genomic DNA
atggataaaaaagaaacccatctgatcgggcatttagaagagcttcgccgccggattatcgtcacccttgcggcattttttctatttctcatcacggcttttttgttcgtacaggacatttatgactggctgatcagggatttggatggaaagctggctgtgctaggaccgagtgaaatcctctgggtgtatatgatgctttccggcatttgtgccattgcggcttctatccctgttgccgcgtaccagctgtggcgtttcgttgcaccggcgctgactaaaacggagcgcaaggtgacgctcatgtacataccaggtttatttgcgttgtttttggcgggcatctccttcggatactttgtcttgtttccgatcgtgctcagctttttgactcatttatcctccggccactttgaaacgatgtttacggctgaccgctactttaggtttatggtgaatttgagcctgccgttcggcttcttgtttgagatgcccttggtggtgatgtttttaacaaggctgggcatcttaaatccttacagactggccaaagcgagaaagctttcctattttctgctgattgtcgtgtccatattgattacaccgcctgattttatttctgattttctcgtgatgatcccgcttcttgtcctgtttgaagtgagtgtcaccctatcggcgtttgtctacaaaaagaggatgagggaagaaacagcggcggccgcttag

SEQ ID NO: 37 - DNA, 174 bp, Bacillus subtilis
  source 1..174: mol_type = genomic DNA
atgccgatcggtcctggaagccttgctgttatcgcaatcgttgctctgattatcttcggtcccaaaaagctgcctgaattggggaaagcagcgggagacacacttcgtgaatttaaaaacgctactaaaggattaacgagtgatgaagaggaaaaaaagaaagaagatcagtaa

SEQ ID NO: 38 - DNA, 765 bp, Bacillus subtilis
  source 1..765: mol_type = genomic DNA
atgacacgaatgaaagtgaatcaaatgtcgctgctggagcatattgctgagcttcgaaaacggttgctgattgtagcgctggcgtttgtcgttttctttattgctggattttttttagcaaagccgattattgtgtatctgcaagaaacagatgaagcgaagcagcttacgcttaacgcgtttaacctgacagacccgctttatgtgtttatgcaatttgcgtttatcatcggcatagtcttgacctcgccggttattctttatcagctttgggcttttgtgagcccgggcctctatgagaaagagcgcaaagtaacgctcagctacattccggtctctattttgctgtttttagcgggcttatctttttcatattatattttatttccttttgttgttgattttatgaagcggatttctcaggacttgaatgtcaatcaggtgatcggaattaatgaatattttcattttcttctgcagctgacgattccgtttggactgctgttccaaatgccggtcatcctcatgtttttgacaaggctcggaattgtgacaccgatgttcttggcgaaaatcagaaagtatgcgtattttacgctgctggtgatcgcagccctgattacaccgcctgagcttctgtcccatatgatggtcacagtcccgcttttgattttatatgaaatcagtatccttatatcgaaggccgcttatcggaaagcacagaaaagcagtgctgccgatcgggacgtgtcttctgggcaataa

SEQ ID NO: 39 - protein, 70 aa, Bacillus subtilis
MFSNIGIPGLILIFVIALIIFGPSKLPEIGRAAGRTLLEFKSATKSLVSGDEKEEKSAELTAVKQDKNAG

SEQ ID NO: 40 - protein, 240 aa, Bacillus subtilis
MDKKETHLIGHLEELRRRIIVTLAAFFLFLITAFLFVQDIYDWLIRDLDGKLAVLGPSEILWVYMMLSGICAIAASIPVAAYQLWRFVAPALTKTERKVTLMYIPGLFALFLAGISFGYFVLFPIVLSFLTHLSSGHFETMFTADRYFRFMVNLSLPFGFLFEMPLVVMFLTRLGILNPYRLAKARKLSYFLLIVVSILITPPDFISDFLVMIPLLVLFEVSVTLSAFVYKKRMREETAA

SEQ ID NO: 41 - protein, 57 aa, Bacillus subtilis
MPIGPGSLAVIAIVALIIFGPKKLPELGKAAGDTLREFKNATKGLTSDEEEKKKEDQ

SEQ ID NO: 42 - protein, 254 aa, Bacillus subtilis
MTRMKVNQMSLLEHIAELRKRLLIVALAFVVFFIAGFFLAKPIIVYLQETDEAKQLTLNAFNLTDPLYVFMQFAFIIGIVLTSPVILYQLWAFVSPGLYEKERKVTLSYIPVSILLFLAGLSFSYYILFPFVVDFMKRISQDLNVNQVIGINEYFHFLLQLTIPFGLLFQMPVILMFLTRLGIVTPMFLAKIRKYAYFTLLVIAALITPPELLSHMMVTVPLLILYEISILISKAAYRKAQKSSAADRDVSSGQ

SEQ ID NO: 43 - DNA, 291 bp, Bifidobacterium longum
  source 1..291: mol_type = genomic DNA
atgcctaatcttcgccccagcgagctcattatcattctgcttatcatcgtgctgctgtttggcgcgaagaagctccctgagctagccaaaagcattggccaatcgatgaagattttccgtgccgagaccaggaccgatgacccggcaacacaacaaaccgtcaatacagtcagcgacgcccctgccccagctccggcggcagcaccggctcccgctcccgccgtaccccaagccgtcacgatgaacgccaccgccgccccgactacagcaaccggagccgaacagcgatga

SEQ ID NO: 44 - DNA, 261 bp, Bifidobacterium longum
  source 1..261: mol_type = genomic DNA
atgttgttcggcatttcgggcacggaactcatggtgattcttgtcatcgctttagtgctggtaggccccgacaagctgcccgactacgcacgcaaggtcggacgatttatccatagcatgcgcgtacgcggccaagcgttgagcgaacaaagcaacatcgacgttcacggccttgtacaggattccggcatcaatgatattcgcaaaggtctggatgatgccacgcaagatgtgaaccggctgctgccgcctatccggtga

SEQ ID NO: 45 - DNA, 1083 bp, Bifidobacterium longum
  source 1..1083: mol_type = genomic DNA
atgagcacggttcccggaaaccctgcgcttccggcaccccttgcaccggcgatgcatcccggcgatcgggatacacatcttgacctcgacgatctcatcgatcactcacacgaggccacgcagcaggccagcgcgggtgcgcaacaccctacacgccggtggaagcggggtgtagggtgcaagtccaaaacgcgcaagccccgcaaccccgatgcggtgatgcctctggccgatcatcttgtcgaatttcgcaaacgctttgttcgggccattgccggcatcatcatcatgtcgatagtgggatggatgttcagcgatcaggtgtttcgtatcctgcaacaaccgttcctgacggcggccgggcagcaacagggactgatgagcatcacattcaatggcgtggtctccgcattcaacgtaaagctggagattgcgttcttccttggtctgacggcctcctgcccgtggtggtcataccaagtgtgggcattcattaatccagggttgaagcgcaaagagcgctggaccgcggttacattcatcggagcctcagtgccgctgttcctcaccggagccggactggcatggtatctgctgccccaagcggtggcgatccttaccggctttgcccccgcaaacaccgccacattgctcagcgccgacgtctattttgatttcattctgcgcatgacagtcgctttcggcctctcattcctgctacccgtagttatggcggcattgacgatgatgaatgcggtcgaaacacgaacatggttgaagcagtggcgtctcgcaacggtcatagcgtttatcttcgcggccgtggccacgccaaccggcgacccaggaacattatgcgcactcgctttgcccatcatcgcaatctatttcgcagccatagccgtatgcgcagtatacgagcacatccagctatggaaagtcatgcgcgcggcgggcgaagaacccaaacttctcaaacttttacataaaatgcgcgccgcgttaccatttcgcgcggcgcgcaaagccaagcgcaccggcaaacaggaagcccctgcaacaataactgcagaaggagaataa

SEQ ID NO: 46 - protein, 96 aa, Bifidobacterium longum
MPNLRPSELIIILLIIVLLFGAKKLPELAKSIGQSMKIFRAETRTDDPATQQTVNTVSDAPAPAPAAAPAPAPAVPQAVTMNATAAPTTATGAEQR

SEQ ID NO: 47 - protein, 86 aa, Bifidobacterium longum
MLFGISGTELMVILVIALVLVGPDKLPDYARKVGRFIHSMRVRGQALSEQSNIDVHGLVQDSGINDIRKGLDDATQDVNRLLPPIR

SEQ ID NO: 48 - protein, 360 aa, Bifidobacterium longum
MSTVPGNPALPAPLAPAMHPGDRDTHLDLDDLIDHSHEATQQASAGAQHPTRRWKRGVGCKSKTRKPRNPDAVMPLADHLVEFRKRFVRAIAGIIIMSIVGWMFSDQVFRILQQPFLTAAGQQQGLMSITFNGVVSAFNVKLEIAFFLGLTASCPWWSYQVWAFINPGLKRKERWTAVTFIGASVPLFLTGAGLAWYLLPQAVAILTGFAPANTATLLSADVYFDFILRMTVAFGLSFLLPVVMAALTMMNAVETRTWLKQWRLATVIAFIFAAVATPTGDPGTLCALALPIIAIYFAAIAVCAVYEHIQLWKVMRAAGEEPKLLKLLHKMRAALPFRAARKAKRTGKQEAPATITAEGE

SEQ ID NO: 49 - protein, 39 aa, Escherichia coli
MNNNDLFQASRRRFLAQLGGLTVAGMLGPSLLTPRRATA

SEQ ID NO: 50 - protein, 27 aa, Escherichia coli
MSLSRRQFIQASGIALCAGAVPLKASA

SEQ ID NO: 51 - protein, 48 aa, Bacillus subtilis
MAYDSRFDEWVQKLKEESFQNNTFDRRKFIQGAGKIAGLSLGLTIAQS

SEQ ID NO: 52 - protein, 49 aa, Streptomyces lividans
MQQDGTQQDRIKQSPAPLNGMSRRGFLGGAGTLALATASGLLLPGTAHA

SEQ ID NO: 53 - protein, 30 aa, Arthrobacter globiformis
MMNLSRRTLLTTGSAATLAYALGMAGSAQA

SEQ ID NO: 54 - DNA, 143 bp, Bacillus subtilis
  source 1..143: mol_type = genomic DNA
taattcctcctttttgttgacattatatcattgatagagttatttgtcaaactagttttttatttggatcccctcgagttcatgaaaaactaaaaaaaatattgacactctatcattgatagagtataattaaaataagcttg

SEQ ID NO: 55 - DNA, 334 bp, Lactococcus lactis
  source 1..334: mol_type = genomic DNA
gtgggtgacaattgattttgatagtcctgatattacttatgatgaatactacggttataaggtcgtggctaatactcatgcagtaatattagatggctacaatgaagcgacaaaagagtttcatgtaactgacccaatcaaagggaaatactggttagctgaatctacggttgcctcagtttacaatgaaacaaatcaatttgcgattgaatttttaaaataaaattagcactctgataaaaagagtgctaatttttttgccaaaagtggaaaaacgtggtaaaatagtgctattgaaaaattgatttagtaaaggaagtgagtaatttagaaa

SEQ ID NO: 56 - DNA, 181 bp, Lactococcus lactis
  source 1..181: mol_type = genomic DNA
attttactacttaagagataaaaaagctagatatatgaaaaaacttattgaaaaaatgcgattaaaggctgataagacttgcatttcaaaacgattttaagtataatgataaggaacggtagattgcaattatgcagactacctataataaaacaaattccccaaaggagacatttttaaa

SEQ ID NO: 57 - DNA, 140 bp, Lactococcus lactis
  source 1..140: mol_type = genomic DNA
aaaacgtttcatacagtttgtaaagagatttttttataaatacgtgatataatgaactagacaacaaatgaacatggtaaaaatattaataacgtttacgtatttttgctgtgtatctcaatttcggaggacagatttaa

SEQ ID NO: 58 - DNA, 193 bp, Lactococcus lactis
  source 1..193: mol_type = genomic DNA
cttttgctcaatattatcttagctgtagccttacaattccctttagaaatcttttacagattaaagaaaagtcatgtaagatacaattagaaagtgttttgtaatcataaagaaatattaaggtggggtaggaatagtataatatgtttattcaaccgaacttaatgggaggaaaaattaaaaaagaacagtt

SEQ ID NO: 59 - DNA, 133 bp, Bifidobacterium longum
  source 1..133: mol_type = genomic DNA
cgcatatcgcggcgcggcgcatctcaatgcgtcgcgccgcacgttaatctgctggcgaaacccagagttctcccagcggccgatgggtatcatgaacgtgcaagccaaccaaagcgatggaagggagtccgtt

SEQ ID NO: 60 - DNA, 240 bp, Bifidobacterium longum
  source 1..240: mol_type = genomic DNA
cttgcatgccgcgcgcttgctcatgatgattcgagacattcctccaaaggagaggaaaaatcacatgtcggttgcgggcaatccgaattgtgagcgctcacaaaaaatacggcatttttgcccaaaacgcacgctgaaacgttgccatgtgtacagagtcggcattacagtagcaactgttggtaaacaatggcccggtgtgccaaagcgcgccaaggccaccctacaagggagaattac

SEQ ID NO: 61 - DNA, 172 bp, Bifidobacterium longum
  source 1..172: mol_type = genomic DNA
cacgcgccactgcatgaagtagccagtgtcttcagtcagcggtaatatcgtataccgctgactgggttctggctcttcaaagtggcacataacccagaaacccagtagaataagcgagttcctgtgcgaaagggtgcaggaaactcacgagacgtccaggaggacaaaagta

SEQ ID NO: 62 - DNA, 3167 bp, synthetic construct
  misc_feature 1..3167: note = pNZ8148 vector
  source 1..3167: mol_type = other DNA
agatctagtcttataactatactgacaatagaaacattaacaaatctaaaacagtcttaattctatcttgagaaagtattggtaataatattattgtcgataacgcgagcataataaacggctctgattaaattctgaagtttgttagatacaatgatttcgttcgaaggaactacaaaataaattataaggaggcactcaccatgggtactgcaggcatgcggtaccactagttctagagagctcaagctttctttgaaccaaaattagaaaaccaaggcttgaaacgttcaattgaaatggcaattaaacaaattacagcacgtgttgctttgattgatagccaaaaagcagcagttgataaagcaattactgatattgctgaaaaattgtaatttataaataaaaatcaccttttagaggtggtttttttatttataaattattcgtttgatttcgctttcgatagaacaatcaaatcgtttctgagacgttttagcgtttatttcgtttagttatcggcataatcgttaaaacaggcgttatcgtagcgtaaaagcccttgagcgtagcgtggctttgcagcgaagatgttgtctgttagattatgaaagccgatgactgaatgaaataataagcgcagcgtccttctatttcggttggaggaggctcaagggagtttgagggaatgaaattccctcatgggtttgattttaaaaattgcttgcaattttgccgagcggtagcgctggaaaatttttgaaaaaaatttggaatttggaaaaaaatggggggaaaggaagcgaattttgcttccgtactacgaccccccattaagtgccgagtgccaatttttgtgccaaaaacgctctatcccaactggctcaagggtttgaggggtttttcaatcgccaacgaatcgccaacgttttcgccaacgttttttataaatctatatttaagtagctttatttttgtttttatgattacaaagtgatacactaattttataaaattatttgattggagttttttaaatggtgatttcagaatcgaaaaaaagagttatgatttctctgacaaaagagcaagataaaaaattaacagatatggcgaaacaaaaagatttttcaaaatctgcggttgcggcgttagctatagaagaatatgcaagaaaggaatcagaacaaaaaaaataagcgaaagctcgcgtttttagaaggatacgagttttcgctacttgtttttgataaggtaattatatcatggctattaaaaatactaaagctagaaattttggatttttattatatcctgactcaattcctaatgattggaaagaaaaattagagagtttgggcgtatctatggctgtcagtcctttacacgatatggacgaaaaaaaagataaagatacatggaatagtagtgatgttatacgaaatggaaagcactataaaaaaccacactatcacgttatatatattgcacgaaatcctgtaacaatagaaagcgttaggaacaagattaagcgaaaattggggaatagttcagttgctcatgttgagatacttgattatatcaaaggttcatatgaatatttgactcatgaatcaaaggacgctattgctaagaataaacatatatacgacaaaaaagatattttgaacattaatgattttgatattgaccgctatataacacttgatgaaagccaaaaaagagaattgaagaatttacttttagatatagtggatgactataatttggtaaatacaaaagatttaatggcttttattcgccttaggggagcggagtttggaattttaaatacgaatgatgtaaaagatattgtttcaacaaactctagcgcctttagattatggtttgagggcaattatcagtgtggatatagagcaagttatgcaaaggttcttgatgctgaaacgggggaaataaaatgacaaacaaagaaaaagagttatttgctgaaaatgaggaattaaaaaaagaaattaaggacttaaaagagcgtattgaaagatacagagaaatggaagttgaattaagtacaacaatagatttattgagaggagggattattgaataaataaaagcccccctgacgaaagtcgacggcaatagttacccttattatcaagataagaaagaaaaggatttttcgctacgctcaaatcctttaaaaaaacacaaaagaccacattttttaatgtggtcttttattcttcaactaaagcacccattagttcaacaaacgaaaattggataaagtgggatatttttaaaatatatatttatgttacagtaatattgacttttaaaaaaggattgattctaatgaagaaagcagacaagtaagcctcctaaattcactttagataaaaatttaggaggcatatcaaatgaactttaataaaattgatttagacaattggaagagaaaagagatatttaatcattatttgaaccaacaaacgacttttagtataaccacagaaattgatattagtgttttataccgaaacataaaacaagaaggatataaattttaccctgcatttattttcttagtgacaagggtgataaactcaaatacagcttttagaactggttacaatagcgacggagagttaggttattgggataagttagagccactttatacaatttttgatggtgtatctaaaacattctctggtatttggactcctgtaaagaatgacttcaaagagttttatgatttatacctttctgatgtagagaaatataatggttcggggaaattgtttcccaaaacacctatacctgaaaatgctttttctctttctattattccttggacttcatttactgggtttaacttaaatatcaataataatagtaattaccttctacccattattacagcaggaaaattcattaataaaggtaattcaatatatttaccgctatctttacaggtacatcattctgtttgtgatggttatcatgctggattgtttatgaactctattcaggaattgtcagataggcctaatgactggcttttataatatgagataatgccgactgtactttttacagtcggttttctaatgtcactaacctgccccgttagttgaagaaggtttttatattacagctcc

SEQ ID NO: 63 - DNA, 4939 bp, synthetic construct
  misc_feature 1..4939: note = pBS423 vector
  source 1..4939: mol_type = other DNA
ggatcctcatcagcaccacccgcgacacgaacgtattacatacgcaatcatatcagtgtcacacatcaggtacaaccgtaccgcaacacgcttcgagcggacgcaagcggcttttgcgcggagcatttccggccatttgcccagcttgttccgcgcttccgagaaggtgtggagttgggttttctgtgatgccgcgcgagcggtctggaggctccgccgaccatggggcatgggtcttcccggcaagccgattcgcaccgcgaatcgagtgattgtagctacaatcacgtcgcttgctactccggccttcggcactcgggttgttgctcctgcgccgaagggcgagggaggctgcgggctcggttcatgtacatgaaccgtctagcttgcttaccttcgatttgatggacatctccatgtggatgtccatggagatgtccatggagatgtccatggagatgtccatggagatgtccatggagatgtccatgtgggtgtccatgtgggtgtccatggatatatccatctgagcgcataggaaaacgcatgagggtggatgatcgttcggggtgatgccttcttccacgaacgggaaggggctcttcctttttctggaatgtcatcttccagcgcccttcgccttgagctccttgagcagcatcgtcgcgttgtcgcggatgctcgcgtccgtgagcggggagagctcgtccgcataggagcggcagaggagcgcgtacacccgttcccgcacccaggcgctgcgcgcgatgcccagcttgaacgcggcccggcacagcatctcgtattcgtcgccggtgagcaggacattgagctggcgtcaaaagttgattagtcatgccgtgtatatacgtccggggtgttttcggccagattccaacagttttgggccactccgggaaggaacagccgacgcttcgctgggctgaaccatctgacttggttcggcgcacgcttgtgcaatgcacaaatgtgcaataggatgtgagctatgagcaacgaatatgtgcaggggacgctggagctgacgcgggcgttcgacggctggtggcttccccagcgtcccctgtgctgcgacgatgactactcccagctggtgcgccggagccgcatcgacgcgctcagatgcaagcacatcgaggcgaatccggcagcgcaggtgaacatgctcgttgttgacgttgattcgtctgagggccgtttaatgagcctgtgggggcatcgggacatgccgcccaacttcatcgcggagaatccggccaacggccactgccacgcgggctgggtgctcaccgaacccgtctgccgcaccgacatggccagactcaagcccctgaagctcctgcacgccgtcaccgaggggctgcgccgcagcgtggacggcgacgagggctattccggcctgctcatgaagaacccgttgagcgacgcgtgggacagcgacctgtgccgcgaggacacctacgacctgcccgacctcgtggccgcgctcgaagcgcacggggacatgccgcccaagagctggacgcgcaccaaacgcgcccgcgaggtcggagtgggccgcaactgcaccctgttcgacgaggcccgcaccctcgcctaccgcgaggtgcgccgactgcctgaccgcacgcccgcctcctccgacctgctgcgcgagtacgtgcgccgcacctgccacgaaatcaacgcctcgttccccgacccgctgcccgtgcgcgaggtcaacgacaccgccaagagcatccacaagtggatcaccacgcgaagccgcatgtggcgagacggtgccgtcgccaacgccgccacgttcgtcgccatccaatccgcacgcggaaagaaatcgggcgaggccagacaaaacgcatttgaagagaagttcgcgcagtacgcgcaggaggtgcttggacaatgaccatccagacaattcgcaagaagcgcccattgcccgccaaggagttagccgaggcctatggggtgtccgtgcgcacgatcaagtactggaattcgcaaacgcgcgaggactggatagacgagcaggcaacgttgcgcgaatccatccgcgcctaccacgacgatgacggccactcgtggagccagaccgccgaacacttcaacatgacccaaggtgccgtgcgccaacgcgcctaccgcgcccgcaaggaacgcgaggccgaggcaaaagccgcaaggccggagtagcaagtgacgtgaacgtatatacgttcactcgattcgcggtgcgaatcggcttgccgggaagacccatgccccatagtcggcagagcctccagaccgctcacgcggcatcgtgccacgactgtggcacatcacgtaacacccgcacatcctcacggtggtgcgcgggtgttacgtgattcgaaccatcggcctgacaggtctcagatcgctccagcgagcttacggcgcatgtactcgctgcggctgatgtggtaccgcctggccatcgcggtcagaccgtccagcgtgctcttgggcatgcggacggacacgctgaccatctgctcgtcgggctcggcgagatggagcccgtagtacacgcgccccgtcaggtcgtccgggacagtctcggactcggccatccgctcatcctccagcacctgctcctcggtcagcccgaccagcgccatcaactgcctgtcgcgttcgctgaaatcactcatagcgtcctcccatcgccgcgcagacggtctatctcgcgcctgaacttcttggtcggcggcgtgaacgcgtggtagatcaccacgaggtcgccgacgaccctgtacagcatctcgacgttcctgccgcgcccgtcgagccctatcgccatccacgcgccggactcgcgctccgcgtccaccatgacgctgcggaacgcggtcaccacgtccttctcggacagttctgggtgacgctccatcaccctgtcaagcacctggatccccgggtaccgagctcgaattctgagcaaaaggccagcaaaaggccagggaccgtaaaaaggccgcgttgctggcgtttttccataggctccgcccccctgacgagcatcacaaaaatcgacgctcaagtcagaggtggcgaaacccgacaggactataaagataccaggcgtttccccctggaagctccctcgtgcgctctcctgttccgaccctgccgcttaccggatacctgtccgcctttctcccttcgggaagcgtggcgctttctcatagctcacgctgtaggtatctcagttcggtgtaggtcgttcgctccaagctgggctgtgtgcacgaaccccccgttcagcccgaccgctgcgccttatccggtaactatcgtcttgagtccaacccggtaagacacgacttatcgccactggcagcagccactggtaacaggattagcagagcgaggtatgtaggcggtgctacagagttcttgaagtggtggcctaactacggctacactagaagaacagtatttggtatctgcgctctgctgaagccagttaccttcggaaaaagagttggtagctcttgatccggcaaacaaaccaccgctggtagcggtggtttttttgtttgcaagcagcagattacgcgcagaaaaaaaggatctcaagaagatcctttgatcttttctacggggtctgacgctcagtggaacgaaaactcacgttaagggattttggccatgagattatcaaaaaggatcttaacctagatccttttaaattaaaaatgaagttttaaatcaatctaaagtatatatgagtactgaattcccattaaataataaaacaaaaaaattaaaaaagtgtttccaccattttttcaatttttttataatttttttaatctgttatttaaatagtttatagttaaatttacattttcattagtccattcaatattctctccaagataactacgaactgctaacaaaattctctccctatgttctaatggagaagactcagccactgcatttcccgcaatatcttttggtatgattttacccgtgtccatagttaaaatcatacggcataaagttaatatagagttggtttcatcatcctgataattatctattaattcctctgacgaatccataatggctcttctcacatcagaaaatggaatatcaggtagtaattcctctaagtcataatttccgtatattcttttattttttcgttttgcttggtaaagcattatggttaaatctgaatttaattccttctgaggaatgtatccttgttcataaagctcttgtaaccattctccataaataaattcttgtttgggaggatgattccacggtaccatttcttgctgaataataattgttaattcaatatatcgtaagttgcttttatctcctattttttttgaaataggtctaattttttgtataagtatttctttactttgatctgtcaatggttcagatacgacgactaaaaagtcaagatcactatttggttttagtccactctcaactcctgatccaaacatgtaagtaccaataaggttattttttaaatgtttccgaagtatttttttcactttattaatttgttcgtatgtattcaaatatatcctcctcactattttgattagtacctattttatatccatagttgttaattaaataaacttaatttagtttatttatagatttcattggcttctaaattttttatctagataataattattttagttaattttattctagattatatatgatatgatctttcatttccataaaactaaagtaagtgtaaacctattcattgttttaaaaatatctcttgccagtcacgttacgttattagttatagttattataacatgtattcacgaacgaaaatcgacctgcaggcatgcaagcttgcatgcctgcaggataggcaggccagctcaag

SEQ ID NO: 64 - DNA, 789 bp, Corynebacterium glutamicum
  source 1..789: mol_type = other DNA
atgacagatttttcatcagcttcaaatgctgatgattcaacacaagatggacgtccaggacgtcgtgctggaaaatcaaaaaaagaatcaaaaccaacaccatggtatattgaaattccagttgttgttgttttaacattagctcttattttcgttttacaaacatttgtcggacgtatgtatatgattccatcaggatcaatggaaccaacattacatggatgtgaaggatgtacaggagatcgtattttagttgaaaaagtttcatattattttacagatccagaaccaggagatgttgttgtattcaaaggaacagattcatggaatgttggattcacaacacaacgttcagataattcagttattcgtggattacaaaatcttggatcatatgttggattagttgctccagatgaaaatgatcttgttaaacgtattattgctacaggtggacaaacagtttcatgtcaagctggagatccaggaattatggttgatggaaaagaagttgatgattcatatacattacaaccagctcaatttccaattgatgaaacatcaggatctacagaatgtggaggaaattattttggaccaattacagttccagatggaaattatttcatgatgggagataatcgtacaaattcaatggattcacgttatcatcttggagatcaatatcaaggaacaattccagaagaaaatattaaaggaaaagttcaagctattattcttccattttcacgtatcggaggagttgatgatccagctattaaaggataa

SEQ ID NO: 65 - DNA, 55 bp, synthetic construct
  misc_feature 1..55: note = primer
  source 1..55: mol_type = other DNA
caatgtcagcgaaaagttaaaggagaaggcatgacagatttttcatcagcttcaa

SEQ ID NO: 66 - DNA, 45 bp, synthetic construct
  misc_feature 1..45: note = primer
  source 1..45: mol_type = other DNA
ttttggttcaaagaaagcttttatcctttaatagctggatcatca

SEQ ID NO: 67 - DNA, 25 bp, synthetic construct
  misc_feature 1..25: note = primer
  source 1..25: mol_type = other DNA
aagctttctttgaaccaaaattaga

SEQ ID NO: 68 - DNA, 24 bp, synthetic construct
  misc_feature 1..24: note = primer
  source 1..24: mol_type = other DNA
ttaacttttcgctgacattggaag

SEQ ID NO: 69 - DNA, 55 bp, synthetic construct
  misc_feature 1..55: note = primer
  source 1..55: mol_type = other DNA
caatgtcagcgaaaagttaaaggagaaggcatgatgaaatttttaaaagaatggg

SEQ ID NO: 70 - DNA, 45 bp, synthetic construct
  misc_feature 1..45: note = primer
  source 1..45: mol_type = other DNA
ttttggttcaaagaaagcttttaaaagaaagaaattttattgagt

SEQ ID NO: 71 - DNA, 171 bp, Lactobacillus reuteri
  source 1..171: mol_type = genomic DNA
tacatttacaaatgaacagatagttgatattatatttaagaattcttcttcagagcctaagattaaagctttcaattggcgaaaagaagttgtacaatatgtataagggtatgtcagtcaccgaatcagatgatctggcattatacttgtaaattatcaggaggttttcat

SEQ ID NO: 72 - protein, 44 aa, Bifidobacterium longum
METNVSRRDFLKGSIVVALGAAGAATLSSCAGGDAAAKADSAVA

SEQ ID NO: 73 - DNA, 132 bp, Bifidobacterium longum
  source 1..132: mol_type = genomic DNA
atggaaacgaacgtctcgcgtcgtgattttcttaagggaagcatcgtggtcgcattgggcgcggccggtgctgctacgctcagctcgtgcgcaggcggcgatgctgcagcgaaagctgattctgcagttgca

SEQ ID NO: 74 - protein, 201 aa, Lactobacillus reuteri
MKAFREAMSWIIPILIGLIIALVIKQFFFQIVRVDGPSMQPNLQNNERVFCLKTAKIHHGSVVVFDANGVDPQVSVKTDYVKRVIGLPGDTVSSRNGNIYVNGKKINQDYISKSQRTTGTGNWTLRSISVQNSWLKNNGATKVPKGEYFVLGDHRSVSNDGRYWGFVPKSKIDGVVKVPSWTGTKTTRENVNKEWQHFYDK

SEQ ID NO: 75 - protein, 216 aa, Bifidobacterium longum
MVGRHSKKARGQSRRYARKPSVWSEIRGYLLTVIAVMLVVLLGRTFVFNVYVIPSRSMEDTLQIGDRVFASRLTPRLFTLHRGDIIVFKDPADWMEGEQLPTNLMSIIDSNRYLIKRVIGLPGDTVACKGSGEPITVNGKPIDESAYLKSGVNPSDSPFSVTVTDGNVFVLGDNRSNSRDSRYHLDDGNNGLVPYDDIQGVALFRFWPFTRIGILN

SEQ ID NO: 76 - DNA, 606 bp, Lactobacillus reuteri
  source 1..606: mol_type = genomic DNA
atgaaagcatttcgtgaagcaatgagttggattattcccattctaatcgggttaataatcgcattagtaattaagcagtttttcttccaaattgttcgggttgatggaccatccatgcaaccaaacttacaaaataatgaacgagtattttgtttgaaaactgccaaaatccatcatggaagtgtcgttgtatttgatgctaatggcgttgatccgcaagtatcagttaaaaccgattatgttaagcgagtaattggacttcctggtgatactgttagctctaggaatggaaatatttatgttaacggcaaaaagattaatcaagactacattagcaaaagtcaacgaacaaccggaactgggaactggacactgcgtagtatctcagttcagaacagttggttaaagaataatggtgccacaaaagttccgaaaggtgaatactttgttcttggggaccaccggagcgtttcaaatgatggtcgttactggggatttgtacctaagagtaagattgatggggttgtaaaagttccatcatggactgggacaaaaacgactcgcgaaaacgttaataaagaatggcagcacttctatgataagtaa

SEQ ID NO: 77 - DNA, 651 bp, Bifidobacterium longum
  source 1..651: mol_type = genomic DNA
atggtggggcgtcatagcaaaaaagcgcgtggccagtcgaggagatatgcgcgaaagccctccgtttggagcgaaattcgcggctatctgctgacagtgatcgcggtgatgctggtcgtgttgctgggacgtaccttcgtgttcaacgtatatgtgattccatcccgcagcatggaagacacgttgcaaatcggcgaccgcgtatttgcctcgcgattgactccgagactctttacactgcaccgtggcgacatcatcgtgttcaaagatcccgcagactggatggagggggagcagcttcccaccaatctgatgtcgataatcgacagcaatcgttacctaatcaaacgtgtcatcggtctgcccggcgataccgtcgcctgcaagggatccggggagcccatcacggtcaacggcaaacccattgatgaaagcgcttatcttaagtccggcgtgaatccaagcgacagccctttttccgtaaccgttactgacggcaacgtgttcgtgcttggtgataatcgctccaattccagagattctcgataccatcttgacgacggcaacaatgggctagtgccatacgacgatatccaaggtgtggcgttgttccgcttctggccatttacgagaatcggcatactgaactga

SEQ ID NO: 78 - protein, 191 aa, Staphylococcus epidermidis
MKKEILEWIVAIAVAIALIAIITKFVGKSYSIKGDSMDPTLKDGERVVVNIIGYKLGGVEKGNVIVFHANKKDDYVKRVIGTPGDSVEYKNDTLYVNGKKQSEPYLNYNEKRKQTEYITGSFKTKNLPNANPQSNVIPKGKYLVLGDNREVSKDSRSFGLIDKDQIVGKVSLRYWPFSEFKSNFNPNNTKN

SEQ ID NO: 79 - DNA, 468 bp, Staphylococcus epidermidis
  source 1..468: mol_type = genomic DNA
atggatcctacattaaaagatggggagcgtgtagtggtaaatattattggctataaattaggtggcgttgaaaaaggaaatgtcattgtatttcatgctaataaaaaagatgattatgttaaaagagttattggaactccaggagatagtgttgaatataaaaatgatacactctatgttaatggtaaaaagcaatcagaaccatacttgaactataatgaaaaacgtaagcaaactgagtatatcacaggtagtttcaaaacaaaaaatttaccaaatgctaatcctcaatctaatgttattcctaaaggtaaatatttagttttgggggataaccgtgaggtaagtaaagatagtcgttcattcggtttaattgacaaagaccaaattgttggaaaggtatcgctcagatattggcctttcagtgaatttaaatctaactttaatccaaataacactaaaaattaa

SEQ ID NO: 80 - DNA, 975 bp, Escherichia coli
  source 1..975: mol_type = genomic DNA
atggcgaatatgtttgccctgattctggtgattgccacactggtgacgggcattttatggtgcgtggataaattctttttcgcacctaaacggcgggaacgtcaggcagcggcgcaggcggctgccggggactcactggataaagcaacgttgaaaaaggttgcgccgaagcctggctggctggaaaccggtgcttctgtttttccggtactggctatcgtattgattgtgcgttcgtttatttatgaaccgttccagatcccgtcaggttcgatgatgccgactctgttaattggtgattttattctggtagagaagtttgcttatggcattaaagatcctatctaccagaaaacgctgatcgaaaccggtcatccgaaacgcggcgatatcgtggtctttaaatatccggaagatccaaagcttgattacatcaagcgcgcggtgggtttaccgggcgataaagtcacttacgatccggtctcaaaagagctgacgattcaaccgggatgcagttccggccaggcgtgtgaaaacgcgctgccggtcacctactcaaacgtggaaccgagcgatttcgttcagaccttctcacgccgtaatggtggggaagcgaccagcggattctttgaagtgccgaaaaacgaaaccaaagaaaatggaattcgtctttccgagcgtaaagagacactgggtgatgtgacgcaccgcattctgacagtgccgattgcgcaggatcaggtggggatgtattaccagcagccagggcaacaactggcaacctggattgttcctccgggacaatacttcatgatgggcgacaaccgcgacaacagcgcggacagccgttactggggctttgtgccggaagcgaatctggtcggtcgggcaacggctatctggatgagcttcgataagcaagaaggcgaatggccgactggtctgcgcttaagtcgcattggcggcatccattaa

SEQ ID NO: 81 - DNA, 555 bp, Bacillus subtilis
  source 1..555: mol_type = genomic DNA
ttgaaatcagaaaatgtttcgaagaaaaagtcaatattagaatgggcaaaagcaattgtgattgctgtcgttcttgctttgctcatccgcaactttatttttgcgccgtatgtcgttgatggtgactctatgtatcctacacttcacaaccgtgaaagggtttttgttaatatgacagtcaaatacatcggcgagtttgatagaggagacatcgtcgtgttaaacggagatgatgttcactatgtcaaacgtattatcggccttcccggcgatacggttgagatgaaaaatgaccagctctatatcaacgggaaaaaggtggacgaaccttatttggcggctaataaaaagagagcgaaacaggacggttttgaccatttgaccgatgatttcggcccggttaaagtgcctgataacaagtattttgtgatgggtgacaatcgtcgcaattccatggacagccgtaacggccttggcctcttcacgaaaaaacaaattgcgggtacgtcaaagtttgttttctacccgtttaacgaaatgcgcaaaacaaattag

SEQ ID NO: 82 - DNA, 582 bp, Bacillus subtilis
  source 1..582: mol_type = genomic DNA
ttgaccgaggaaaaaaatacgaatactgagaaaacggcgaagaaaaaaaccaatacgtacctggaatggggtaaagcgattgtcatcgctgttctgctggctctcctgatccgtcactttttgtttgaaccgtatttagttgaaggttcatctatgtatcccacattacatgacggagaaaggctgtttgtgaataaaacagtcaactatatcggcgagctgaagcgcggagatatcgttattatcaacggtgaaacttctaaaatccattatgtaaaaagattgatcggaaagcctggagaaaccgttcaaatgaaggatgacacgctttatataaacggtaaaaaagtagccgagccttacttgtctaaaaacaagaaggaagcagaaaaacttggtgtcagtctgacaggagactttggaccggttaaggttccgaaaggcaaatactttgtcatgggagataaccggctgaattctatggacagccgaaacgggctgggactgatcgcggaagatcgaattgtcggcacatcgaagtttgtctttttcccgtttaacgaaatgcgtcaaacaaaataa

SEQ ID NO: 83 - DNA, 789 bp, Corynebacterium glutamicum
  source 1..789: mol_type = genomic DNA
gtgactgatttttctagtgcttcaaatgctgacgattccacgcaggacggtcgtcctggtcgacgtgctggaaagtctaagaaggaatcgaagccaactccgtggtacatcgaaattccagtggttgtggttctgaccctcgcgctgattttcgtgctccagacgtttgtcggacgcatgtacatgattccgagtggttcgatggaacctactttgcacggatgtgagggctgcacgggtgaccgcatcctggtggagaaggtttcttactacttcacggatccagagccgggcgatgttgtggtgttcaagggtactgattcctggaacgttggattcactacgcagcgttccgataattcggtgatccgcggcctgcagaacctgggttcttacgtgggtcttgtcgcacctgatgaaaatgacctggtcaagcgcattatcgccaccggcggtcagactgtttcgtgccaagccggtgatcctggaatcatggttgacggcaaggaagtcgatgacagctacacgctgcaacctgcgcaattccccatcgatgagacctccggttccaccgaatgcggcggcaactatttcggccccatcaccgtgcctgacggcaactacttcatgatgggtgacaaccgcaccaactccatggattcccgctaccacctgggcgatcagtaccaaggaaccatccctgaggaaaacatcaagggcaaagttcaagcaattatcctgccatttagccgaatcggtggcgtcgacgaccctgccatcaaaggctag

SEQ ID NO: 84 - DNA, 627 bp, Lactococcus lactis
  source 1..627: mol_type = genomic DNA
atgatgaaatttttaaaagaatggggattatttatctttataattgccgctgtccttctctcgcgcgtctttatttggtcactagttgtcgttgatggccattcaatggaccctactttagccgataaagaaagacttgtaattgttagaacgacaaaaattaatcgttttgatattgtagttgctaaagaaaacgcggctgatggttcaaccaaagatattgtcaaacgtgtcgttgggatgcctggggacactataaaattcgaccatgaccaacttactatcaataataaggtttatccagaaaactatctcaaagactatcaaaaacaattggctgatggtcaattggaaaaaacttacgggaactatcctttgacaaaagcattaactgatcaaaatcgtagtttatttgtaagcttagctcagagcaccaaagcttttacaacggatagtactggtaatccaacctttacagtcaaagtccctgacggacaatacttcttgatgggagataatcgtgttgtgtctcaagatagccgagcagttggaagtttcaaacgttcagcgattattggtgaagccaaattacgagtttggccactcaataaaatttctttcttttaa

SEQ ID NO: 85 - DNA, 918 bp, synthetic construct
  source 1..918: mol_type = other DNA
gattcaaatggcaatcaagaaatcaacggaaaagaaaaattaagcgttaatgatagtaagttgaaggattttggtaagacagttccggttggtattgacgaagaaaatggtatgataaaagtaagctttatgcttactgcgcaattctatgaaattaaacctaccaaagaaaatgagcaatatattggtatgcttcgccaagctgttaaaaatgaatctccagtccacatttttttaaaaccaaactcaaatgaaatcgggaaagttgagagcgcaagtccagaggacgtaagatatttcaagacgattttaactaaagaagtaaaaggacagacaaacaaattggcgagtgtcattccagatgtagctacattaaactcattgttcaatcaaattaaaaaccaatcttgtggtacttctactgcttcaagtccatgcattacttttcgatatccagtagacgggtgttatgcacgtgcccataaaatgcgtcaaatattgatgaataatggctatgattgtgaaaaacaatttgtgtatggtaacttaaaagcatctactggaacctgttgtgttgcatggagctatcatgttgcaattttggttagttacaaaaatgcttctggagtgacggaaaaacgtattattgatccatcacttttttcaagcggtcctgtgacagatacagcctggagaaatgcttgcgttaatacatcttgcggctctgcttcagttagttcatatgctaataccgcaggaaatgtttactatcgatctcccagtaattcttacttgtatgataacaatcttatcaatacaaactgtgtcttgactaagttttcattactttcaggatgttctccttcacctgcccctgatgtctcaagttgtggatttcatcatcaccatcatcattaa

SEQ ID NO: 86 - DNA, 42 bp, synthetic construct
  source 1..42: mol_type = other DNA
  misc_feature 1..42: note = primer
cgtcgtgccaccgcagattcaaatggcaatcaagaaatcaac

SEQ ID NO: 87 - DNA, 42 bp, synthetic construct
  source 1..42: mol_type = other DNA
  misc_feature 1..42: note = primer
atcatgccttctcctttaatgatgatggtgatgatgaaatcc

SEQ ID NO: 88 - DNA, 29 bp, synthetic construct
  source 1..29: mol_type = other DNA
  misc_feature 1..29: note = primer
aggagaaggcatgatgaaatttttaaaag

SEQ ID NO: 89 - DNA, 22 bp, synthetic construct
  source 1..22: mol_type = other DNA
  misc_feature 1..22: note = primer
tgcggtggcacgacgaggagtc

SEQ ID NO: 90 - DNA, 25 bp, synthetic construct
  source 1..25: mol_type = other DNA
  misc_feature 1..25: note = primer
cttttgctcaatattatcttagctg

SEQ ID NO: 91 - DNA, 25 bp, synthetic construct
  source 1..25: mol_type = other DNA
  misc_feature 1..25: note = primer
aactgttcttttttaatttttcctc

SEQ ID NO: 92 - DNA, 39 bp, synthetic construct
  source 1..39: mol_type = other DNA
  misc_feature 1..39: note = primer
taaaaaagaacagttgcatgcggtaccactagtatgcca

SEQ ID NO: 93 - DNA, 41 bp, synthetic construct
  source 1..41: mol_type = other DNA
  misc_feature 1..41: note = primer
aatattgagcaaaagagatctggagctgtaatataaaaacc